European Patent Specification EP 3 727 426 B1, published November 26, 2025. Title: INCRETIN ANALOGS AND USES THEREOF. Applicant: Eli Lilly and Company. The sequence listing filed with the application follows.

SEQUENCE LISTING (27 sequences)

SEQ ID NO: 1 - protein, 29 aa, Homo sapiens
HSQGTFTSDYSKYLDSRRAQDFVQWLMNT

SEQ ID NO: 2 - protein, 30 aa, Homo sapiens
HAEGTFTSDVSSYLEGQAAKEFIAWLVKGR

SEQ ID NO: 3 - protein, 37 aa, Homo sapiens
HSQGTFTSDYSKYLDSRRAQDFVQWLMNTKRNRNNIA

SEQ ID NO: 4 - protein, 42 aa, Homo sapiens
YAEGTFISDYSIAMDKIHQQDFVNWLLAQKGKKNDWKHNITQ

SEQ ID NO: 5 - protein, 39 aa, Artificial Sequence
  Synthetic Construct
  MISC_FEATURE (2)..(2): Xaa at position 2 is Aib
  MISC_FEATURE (13)..(13): Xaa at position 13 is Leu or alpha-methyl-Leu
  MISC_FEATURE (17)..(17): Xaa at position 17 is any amino acid with a functional group available for conjugation wherein the functional group is conjugated to a C16-C22 fatty acid
  MISC_FEATURE (19)..(19): Xaa at position 19 is Gln or Ala
  MISC_FEATURE (20)..(20): Xaa at position 20 is Aib, alpha-methyl-Lys, Gln, or His
  MISC_FEATURE (28)..(28): Xaa at position 28 is Glu or Ala
  MISC_FEATURE (29)..(29): Xaa at position 29 is Gly or Aib
  MISC_FEATURE (34)..(34): Xaa at position 34 is Gly or Aib
YXQGTFTSDYSIXLDKXAXXAFIEYLLXXGPSSXAPPPS

SEQ ID NO: 6 - protein, 39 aa, Artificial Sequence
  Synthetic Construct
  MISC_FEATURE (2)..(2): Xaa at position 2 is alpha-amino-isobutyric acid
  MISC_FEATURE (13)..(13): Xaa at position 13 is alpha-methyl-Leu
  MISC_FEATURE (17)..(17): Lys at position 17 is modified with (2-[2-(2-Amino-ethoxy)-ethoxy]-acetyl)-(gamma-Glu)-CO-(CH2)18-HCO 2H
  MISC_FEATURE (29)..(29): Xaa at position 29 is alpha-amino-isobutyric acid
  MOD_RES (39)..(39): Ser at position 39 is optionally amidated
YXQGTFTSDYSIXLDKKAQHAFIEYLLAXGPSSGAPPPS

SEQ ID NO: 7 - protein, 39 aa, Artificial Sequence
  Synthetic Construct
  MISC_FEATURE (2)..(2): Xaa at position 2 is alpha-amino-isobutyric acid
  MISC_FEATURE (13)..(13): Xaa at position 13 is alpha-methyl-Leu
  MOD_RES (17)..(17): Lys at position 17 is chemically modified by conjugation of the epsilon-amino group of the Lys side chain with (2-[2-(2-Amino-ethoxy)-ethoxy]-acetyl)2-(gamma-Glu)-CO-(CH2)18-CO 2H)
  MISC_FEATURE (20)..(20): Xaa at position 20 is alpha-methyl-Lys
  MISC_FEATURE (29)..(29): Xaa at position 29 is alpha-amino-isobutyric acid
  MOD_RES (39)..(39): Ser at position 39 is optionally amidated
YXQGTFTSDYSIXLDKKAQXAFIEYLLAXGPSSGAPPPS

SEQ ID NO: 8 - protein, 39 aa, Artificial Sequence
  Synthetic Construct
  MISC_FEATURE (2)..(2): Xaa at position 2 is 2-aminoisobutyric acid
  MISC_FEATURE (13)..(13): Xaa at position 13 is alpha-methyl-Leu
  MOD_RES (17)..(17): Lys at position 17 is chemically modified by conjugation of the epsilon-amino group of the Lys side chain with (2-[2-(2-Amino-ethoxy)-ethoxy]-acetyl)2-(gamma-Glu)-CO-(CH2)18-CO 2H)
  MISC_FEATURE (20)..(20): Xaa at position 20 is alpha-methyl-Lys
  MOD_RES (39)..(39): Ser at position 39 is optionally amidated
YXQGTFTSDYSIXLDKKAQXAFIEYLLEGGPSSGAPPPS

SEQ ID NO: 9 - protein, 39 aa, Artificial Sequence
  Synthetic Construct
  MISC_FEATURE (2)..(2): Xaa at position 2 is 2-aminoisobutyric acid
  MOD_RES (17)..(17): Lys at position 17 is chemically modified by conjugation of the epsilon-amino group of the Lys side chain with (2-[2-(2-Amino-ethoxy)-ethoxy]-acetyl)-(gamma-Glu)-CO-(CH2)18-CO2 H
  MISC_FEATURE (20)..(20): Xaa at position 20 is alpha-amino-isobutyric acid
  MISC_FEATURE (29)..(29): Xaa at position 29 is alpha-amino-isobutyric acid
  MOD_RES (39)..(39): Ser at position 39 is optionally amidated
YXQGTFTSDYSILLDKKAQXAFIEYLLAXGPSSGAPPPS

SEQ ID NO: 10 - protein, 39 aa, Artificial Sequence
  Synthetic Construct
  MISC_FEATURE (2)..(2): Xaa at position 2 is alpha-amino-isobutyric acid
  MISC_FEATURE (13)..(13): Xaa at position 13 is alpha-methyl-Leu
  MOD_RES (17)..(17): Lys at position 17 is chemically modified by conjugation of the epsilon-amino group of the Lys side chain with (2-[2-(2-Amino-ethoxy)-ethoxy]-acetyl)2-(gamma-Glu)-CO-(CH2)18-CO 2H
  MISC_FEATURE (29)..(29): Xaa at position 29 is alpha-amino-isobutyric acid
  MOD_RES (39)..(39): Ser at position 39 is optionally amidated
YXQGTFTSDYSIXLDKKAAQAFIEYLLEXGPSSGAPPPS

SEQ ID NO: 11 - protein, 39 aa, Artificial Sequence
  Synthetic Construct
  MISC_FEATURE (2)..(2): Xaa at position 2 is alpha-amino-isobutyric acid
  MISC_FEATURE (13)..(13): Xaa at position 13 is alpha-methyl-Leu
  MOD_RES (17)..(17): Lys at position 17 is chemically modified by conjugation of the epsilon-amino group of the Lys side chain with (2-[2-(2-Amino-ethoxy)-ethoxy]-acetyl)2-(gamma-Glu)-CO-(CH2)18-CO 2H
  MOD_RES (39)..(39): Ser at position 39 is optionally amidated
YXQGTFTSDYSIXLDKKAAQAFIEYLLEGGPSSGAPPPS

SEQ ID NO: 12 - protein, 39 aa, Artificial Sequence
  Synthetic Construct
  MISC_FEATURE (2)..(2): Xaa at position 2 is alpha-amino-isobutyric acid
  MISC_FEATURE (13)..(13): Xaa at position 13 is alpha-methyl-Leu
  MOD_RES (17)..(17): Lys at position 17 is chemically modified by conjugation of the epsilon-amino group of the Lys side chain with (2-[2-(2-Amino-ethoxy)-ethoxy]-acetyl)2-(gamma-Glu)-CO-(CH2)18-CO 2H
  MOD_RES (39)..(39): Ser at position 39 is optionally amidated
YXQGTFTSDYSIXLDKKAQHAFIEYLLEGGPSSGAPPPS

SEQ ID NO: 13 - protein, 39 aa, Artificial Sequence
  Synthetic Construct
  MISC_FEATURE (2)..(2): Xaa at position 2 is alpha-amino-isobutyric acid
  MOD_RES (17)..(17): Lys at position 17 is chemically modified by conjugation of the epsilon-amino group of the Lys side chain with (2-[2-(2-Amino-ethoxy)-ethoxy]-acetyl)2-(gamma-Glu)-CO-(CH2)18-CO 2H
  MISC_FEATURE (20)..(20): Xaa at position 20 is alpha-methyl-Lys
  MOD_RES (39)..(39): Ser at position 39 is optionally amidated
YXQGTFTSDYSILLDKKAQXAFIEYLLEGGPSSGAPPPS

SEQ ID NO: 14 - protein, 39 aa, Artificial Sequence; identical to SEQ ID NO: 12
  Synthetic Construct
  MISC_FEATURE (2)..(2): Xaa at position 2 is alpha-amino-isobutyric acid
  MISC_FEATURE (13)..(13): Xaa at position 13 is alpha-methyl-Leu
  MOD_RES (17)..(17): Lys at position 17 is chemically modified by conjugation of the epsilon-amino group of the Lys side chain with (gamma-Glu)2-CO-(CH2)18-CO2H
  MOD_RES (39)..(39): Ser at position 39 is optionally amidated

SEQ ID NO: 15 - protein, 39 aa, Artificial Sequence; identical to SEQ ID NO: 12
  Synthetic Construct
  MISC_FEATURE (2)..(2): Xaa at position 2 is alpha-amino-isobutyric acid
  MISC_FEATURE (13)..(13): Xaa at position 13 is alpha-methyl-Leu
  MOD_RES (17)..(17): Lys at position 17 is chemically modified by conjugation of the epsilon-amino group of the Lys side chain with (2-[2-(2-Amino-ethoxy)-ethoxy]-acetyl)-(gamma-Glu)-CO-(CH2)18-CO2 H
  MOD_RES (39)..(39): Ser at position 39 is optionally amidated

SEQ ID NO: 16 - protein, 39 aa, Artificial Sequence; identical to SEQ ID NO: 8
  Synthetic Consruct
  MISC_FEATURE (2)..(2): Xaa at position 2 is alpha-amino-isobutyric acid
  MISC_FEATURE (13)..(13): Xaa at position 13 is alpha-methyl-Leu
  MOD_RES (17)..(17): Lys at position 17 is chemically modified by conjugation of the epsilon-amino group of the Lys side chain with (2-[2-(2-Amino-ethoxy)-ethoxy]-acetyl)2-(gamma-Glu)-CO-(CH2)18-CO 2H
  MISC_FEATURE (20)..(20): Xaa at position 20 is alpha-amino-isobutyric acid
  MOD_RES (39)..(39): Ser at position 39 is optionally amidated

SEQ ID NO: 17 - protein, 39 aa, Artificial Sequence; identical to SEQ ID NO: 8
  Synthetic Construct
  MISC_FEATURE (2)..(2): Xaa at position 2 is alpha-amino-isobutyric acid
  MISC_FEATURE (13)..(13): Xaa at position 2 is alpha-methyl-leucine
  MOD_RES (17)..(17): Lys at position 17 is chemically modified by conjugation of the epsilon-amino group of the Lys side chain with (2-[2-(2-Amino-ethoxy)-ethoxy]-acetyl)-(gamma-Glu)-CO-(CH2)18-CO2 H
  MISC_FEATURE (20)..(20): Xaa at position 20 is alpha-amino-isobutyric acid
  MOD_RES (39)..(39): Ser at position 39 is optionally amidated

SEQ ID NO: 18 - protein, 39 aa, Artificial Sequence
  Synthetic Construct
  MISC_FEATURE (2)..(2): Xaa at position 2 is alpha-amino-isobutyric acid
  MISC_FEATURE (13)..(13): Xaa at position 13 is alpha-methyl-Leu
  MOD_RES (17)..(17): Lys at position 17 is chemically modified by conjugation of the epsilon-amino group of the Lys side chain with (2-[2-(2-Amino-ethoxy)-ethoxy]-acetyl)-(gamma-Glu)-CO-(CH2)18-CO2 H
  MISC_FEATURE (20)..(20): Xaa at position 20 is alpha-amino-isobutyric acid
  MISC_FEATURE (29)..(29): Xaa at position 29 is alpha-amino-isobutyric acid
  MOD_RES (39)..(39): Ser at position 39 is optionally amidated
YXQGTFTSDYSIXLDKKAQXAFIEYLLEXGPSSGAPPPS

SEQ ID NO: 19 - protein, 39 aa, Artificial Sequence
  Synthetic Construct
  MISC_FEATURE (2)..(2): Xaa at position 2 is alpha-amino-isobutyric acid
  MISC_FEATURE (13)..(13): Xaa at position 13 is alpha-methyl-Leu
  MOD_RES (17)..(17): Lys at position 17 is chemically modified by conjugation of the epsilon-amino group of the Lys side chain with (2-[2-(2-Amino-ethoxy)-ethoxy]-acetyl)-(gamm-Glu)-CO-(CH2)18-CO2H
  MISC_FEATURE (20)..(20): Xaa at position 20 is alpha-amino-isobutyric acid
  MISC_FEATURE (29)..(29): Xaa at position 29 is alpha-amino-isobutyric acid
  MISC_FEATURE (34)..(34): Xaa at position 34 is alpha-amino-isobutyric acid
  MOD_RES (39)..(39): Ser at position 39 is optionally amidated
YXQGTFTSDYSIXLDKKAQXAFIEYLLEXGPSSXAPPPS

SEQ ID NO: 20 - protein, 39 aa, Artificial Sequence; identical to SEQ ID NO: 9
  Synthetic Construct
  MISC_FEATURE (2)..(2): Xaa at position 2 is alpha-amino-isobutyric acid
  MOD_RES (17)..(17): Lys at position 17 is chemically modified by conjugation of the epsilon-amino group of the Lys side chain with (2-[2-(2-Amino-ethoxy)-ethoxy]-acetyl)2-(gamma-Glu)-CO-(CH2)18-CO 2H
  MISC_FEATURE (20)..(20): Xaa at position 20 is alpha-amino-isobutyric acid
  MISC_FEATURE (29)..(29): Xaa at position 29 is alpha-amino-isobutyric acid
  MOD_RES (39)..(39): Ser at position 39 is optionally amidated

SEQ ID NO: 21 - protein, 39 aa, Artificial Sequence; identical to SEQ ID NO: 13
  Synthetic Construct
  MISC_FEATURE (2)..(2): Xaa at position 2 is alpha-amino-isobutyric acid
  MOD_RES (17)..(17): Lys at position 17 is chemically modified by conjugation of the epsilon-amino group of the Lys side chain with (2-[2-(2-Amino-ethoxy)-ethoxy]-acetyl)2-(gamma-Glu)-CO-(CH2)18-CO 2H
  MISC_FEATURE (20)..(20): Xaa at position 20 is alpha-amino-isobutyric acid
  MOD_RES (39)..(39): Ser at position 39 is optionally amidated

SEQ ID NO: 22 - protein, 39 aa, Artificial Sequence
  Synthetic Construct
  MISC_FEATURE (2)..(2): Xaa at position 2 is alpha-amino-isobutyric acid
  MOD_RES (17)..(17): Lys at position 17 is chemically modified by conjugation of the epsilon-amino group of the Lys side chain with (2-[2-(2-Amino-ethoxy)-ethoxy]-acetyl)2-(gamma-Glu)-CO-(CH2)18-CO 2H
  MISC_FEATURE (20)..(20): Xaa at position 20 is alpha-amino-isobutyric acid
  MISC_FEATURE (29)..(29): Xaa at position 29 is alpha-amino-isobutyric acid
  MOD_RES (39)..(39): Ser at position 39 is optionally amidated
YXQGTFTSDYSILLDKKAQXAFIEYLLEXGPSSGAPPPS

SEQ ID NO: 23 - protein, 39 aa, Artificial Sequence; identical to SEQ ID NO: 13
  Synthetic Construct
  MISC_FEATURE (2)..(2): Xaa at position 2 is alpha-amino-isobutyric acid
  MOD_RES (17)..(17): Lys at position 17 is chemically modified by conjugation of the epsilon-amino group of the Lys side chain with (2-[2-(2-Amino-ethoxy)-ethoxy]-acetyl)-(gamma-Glu)-CO-(CH2)18-CO2 H
  MISC_FEATURE (20)..(20): Xaa at position 20 is alpha-amino-isobutyric acid
  MOD_RES (39)..(39): Ser at position 39 is optionally amidated

SEQ ID NO: 24 - protein, 39 aa, Artificial Sequence; identical to SEQ ID NO: 22
  Synthetic Construct
  MISC_FEATURE (2)..(2): Xaa at position 2 is alpha-amino-isobutyric acid
  MOD_RES (17)..(17): Lys at position 17 is chemically modified by conjugation of the epsilon-amino group of the Lys side chain with (2-[2-(2-Amino-ethoxy)-ethoxy]-acetyl)-(gamma-Glu)2-CO-(CH2)18-CO 2H
  MISC_FEATURE (20)..(20): Xaa at position 20 is alpha-amino-isobutyric acid
  MISC_FEATURE (29)..(29): Xaa at position 29 is alpha-amino-isobutyric acid
  MOD_RES (39)..(39): Ser at position 39 is optionally amidated

SEQ ID NO: 25 - protein, 39 aa, Artificial Sequence; identical to SEQ ID NO: 22
  Synthetic Construct
  MISC_FEATURE (2)..(2): Xaa at position 2 is alpha-amino-isobutyric acid
  MOD_RES (17)..(17): Lys at position 17 is chemically modified by conjugation of the epsilon-amino group of the Lys side chain with (2-[2-(2-Amino-ethoxy)-ethoxy]-acetyl)-(gamma-Glu)-CO-(CH2)18-CO2 H
  MISC_FEATURE (20)..(20): Xaa at position 20 is alpha-amino-isobutyric acid
  MISC_FEATURE (29)..(29): Xaa at position 29 is alpha-amino-isobutyric acid
  MOD_RES (39)..(39): Ser at position 39 is optionally amidated

SEQ ID NO: 26 - protein, 10 aa, Artificial Sequence
  Synthetic Construct
GPSSGAPPPS

SEQ ID NO: 27 - protein, 10 aa, Artificial Sequence
  Synthetic Construct
  MISC_FEATURE (5)..(5): Xaa at position 5 is alpha-amino-isobutyric acid
GPSSXAPPPS